European Patent Application EP 4 382 119 A1, published June 12, 2024. Title: A kit for use in the treatment of hematological cancer. Applicant: AvenCell Europe GmbH. Application EP. The sequence listing filed with the application follows.

SEQUENCE LISTING (56 sequences)

SEQ ID NO: 1 - protein, 5 aa, synthetic construct
  source 1..5: note = linker
GGGGS

SEQ ID NO: 2 - protein, 25 aa, synthetic construct
  source 1..25: note = linker
GGGGSGGGGSGASAAGGGGSGGGGS

SEQ ID NO: 3 - protein, 25 aa, synthetic construct
  source 1..25: note = Linker
GGGGSGGGGSGGGGSGGGGSGGGGS

SEQ ID NO: 4 - protein, 119 aa, Mus musculus
EVQLQQSGPELVKPGASVKMSCKASGYTFTDYYMKWVKQSHGKSLEWIGDIIPSNGATFYNQKFKGKATLTVDRSSSTAYMHLNSLTSEDSAVYYCTRSHLLRASWFAYWGQGTLVTVS

SEQ ID NO: 5 - protein, 113 aa, Mus musculus
DFVMTQSPSSLTVTAGEKVTMSCKSSQSLLNSGNQKNYLTWYLQKPGQPPKLLIYWASTRESGVPDRFTGSGSGTDFTLTISSVQAEDLAVYYCQNDYSYPYTFGGGTKLEIK

SEQ ID NO: 6 - protein, 250 aa, synthetic construct
  source 1..250: note = anti-CD123 scFv
EVQLQQSGPELVKPGASVKMSCKASGYTFTDYYMKWVKQSHGKSLEWIGDIIPSNGATFYNQKFKGKATLTVDRSSSTAYMHLNSLTSEDSAVYYCTRSHLLRASWFAYWGQGTLVTVSAASGGGGSGGGGSGGGGSDFVMTQSPSSLTVTAGEKVTMSCKSSQSLLNSGNQKNYLTWYLQKPGQPPKLLIYWASTRESGVPDRFTGSGSGTDFTLTISSVQAEDLAVYYCQNDYSYPYTFGGGTKLEIK

SEQ ID NO: 7 - protein, 112 aa, synthetic construct
  source 1..112: note = Humanized scFv VL chain
  VARIANT 24: note = X can be any amino acid
DIVMTQSPDSLAVSLGERATINCXSSQSLLNSRTXKNYLAWYQQKPGQPPKLLIYWASTRXSGVPDRFSGSGSGTDFTLTISSLQAEDVAVYYCKQSYNLXTFGGGTKVEIK

SEQ ID NO: 8 - protein, 112 aa, synthetic construct
  source 1..112: note = Humanized scFv VL chain
DIVMTQSPDSLAVSLGERATINCKSSQSLLNSRTPKNYLAWYQQKPGQPPKLLIYWASTRKSGVPDRFSGSGSGTDFTLTISSLQAEDVAVYYCKQSYNLLTFGGGTKVEIK

SEQ ID NO: 9 - protein, 120 aa, synthetic construct
  source 1..120: note = Humanized scFv VH chain
QVQLVQSGAEVKKPGASVKVSCKASGYTFTHYYIYWVRQAPGQGLEWMGGVNPSNGGTHFNEKFKSRVTMTRDTSISTAYMELSRLRSDDTAVYYCARSEYDYGLGFAYWGQGTLVTVSS

SEQ ID NO: 10 - protein, 526 aa, synthetic construct
  source 1..526: note = Targeting module
GQVQLVQSGAEVKKPGSSVKVSCKASGYTFTDYYIHWVRQAPGQGLEWMGDIIPSNGATFYNQRFKGRVTITADESTSTAYMELSSLRSEDTAVYYCTRSHLLRASWFAYWGQGTLVTVSSASGGGGSGGGGSGGGGSDIVMTQTPLSLSVTPGQPASISCRSSQSLLNSGNQKNYLTWYLQKPGQSPQLLIYWASTRFIGVPDRFSGSGSGTDFTLKISRVEAEDVGVYYCQNDYSYPYTFGQGTKLEIKAAARGDIVMTQSPDSLAVSLGERATINCKSSQSLLNSRTPKNYLAWYQQKPGQPPKLLIYWASTRKSGVPDRFSGSGSGTDFTLTISSLQAEDVAVYYCKQSYNLLTFGGGTKVEIKGGGGSGGGGSGASAAGGGGSGGGGSQVQLVQSGAEVKKPGASVKVSCKASGYTFTHYYIYWVRQAPGQGLEWMGGVNPSNGGTHFNEKFKSRVTMTRDTSISTAYMELSRLRSDDTAVYYCARSEYDYGLGFAYWGQGTLVTVSSGGGGSHHHHHHHH

SEQ ID NO: 11 - protein, 526 aa, synthetic construct
  source 1..526: note = Targeting module
GQVQLVQSGAEVKKPGASVKMSCKASGYTFTDYYMKWVKQAPGQGLEWIGDIIPSNGATFYNQKFQGRATLTVDTSTSTAYMELSSLRSEDTAVYYCTRSHLLRASWFAYWGQGTLVTVSSASGGGGSGGGGSGGGGSDIVMTQSPDSLAVSLGERATINCKSSQSLLNSGNQKNYLTWYLQKPGQPPKLLIYWASTRESGVPDRFSGSGSGTDFTLTISSVQAEDVAVYYCQNDYSYPYTFGGGTKLEIKAAARGDIVMTQSPDSLAVSLGERVTMNCKSSQSLLNSRTPKNYLAWYQQKPGQSPKLLIYWASTRKSGVPDRFSGSGSGTDFTLTISSVQAEDVAVYYCKQSYNLLTFGGGTKLEIKGGGGSGGGGSGASAAGGGGSGGGGSQVQLVESGAEVVKPGASVKLSCKASGYAFTHYYIYWIKQAPGQGLEWIGGVNPSNGGTHFNEKFKSRATLTVDTSISTAYMELSRLRSDDTAVYYCTRSEYDYGLGFAYWGQGTLVTVSSGGGGSHHHHHHHH

SEQ ID NO: 12 - protein, 525 aa, synthetic construct
  source 1..525: note = Targeting module
EVQLQQSGPELVKPGASVKMSCKASGYTFTDYYMKWVKQSHGKSLEWIGDIIPSNGATFYNQKFKGKATLTVDRSSSTAYMHLNSLTSEDSAVYYCTRSHLLRASWFAYWGQGTLVTVSAASGGGGSGGGGSGGGGSDFVMTQSPSSLTVTAGEKVTMSCKSSQSLLNSGNQKNYLTWYLQKPGQPPKLLIYWASTRESGVPDRFTGSGSGTDFTLTISSVQAEDLAVYYCQNDYSYPYTFGGGTKLEIKAAARGDIVMTQSPDSLAVSLGERATINCKSSQSLLNSRTPKNYLAWYQQKPGQPPKLLIYWASTRKSGVPDRFSGSGSGTDFTLTISSLQAEDVAVYYCKQSYNLLTFGGGTKVEIKGGGGSGGGGSGASAAGGGGSGGGGSQVQLVQSGAEVKKPGASVKVSCKASGYTFTHYYIYWVRQAPGQGLEWMGGVNPSNGGTHFNEKFKSRVTMTRDTSISTAYMELSRLRSDDTAVYYCARSEYDYGLGFAYWGQGTLVTVSSGGGGSHHHHHHHH

SEQ ID NO: 13 - protein, 525 aa, synthetic construct
  source 1..525: note = Targeting module
EVQLQQSGPELVKPGASVKMSCKASGYTFTDYYMKWVKQSHGKSLEWIGDIIPSNGATFYNQKFKGKATLTVDRSSSTAYMHLNSLTSEDSAVYYCTRSHLLRASWFAYWGQGTLVTVSAASGGGGSGGGGSGGGGSDFVMTQSPSSLTVTAGEKVTMSCKSSQSLLNSGNQKNYLTWYLQKPGQPPKLLIYWASTRESGVPDRFTGSGSGTDFTLTISSVQAEDLAVYYCQNDYSYPYTFGGGTKLEIKAAARGDIVMTQSPDSLAVSLGERVTMNCKSSQSLLNSRTPKNYLAWYQQKPGQSPKLLIYWASTRKSGVPDRFSGSGSGTDFTLTISSVQAEDVAVYYCKQSYNLLTFGGGTKLEIKGGGGSGGGGSGASAAGGGGSGGGGSQVQLVESGAEVVKPGASVKLSCKASGYAFTHYYIYWIKQAPGQGLEWIGGVNPSNGGTHFNEKFKSRATLTVDTSISTAYMELSRLRSDDTAVYYCTRSEYDYGLGFAYWGQGTLVTVSSGGGGSHHHHHHHH

SEQ ID NO: 14 - protein, 526 aa, synthetic construct
  source 1..526: note = Targeting module
GQVQLVQSGAEVKKPGASVKMSCKASGYTFTDYYMKWVKQAPGQGLEWIGDIIPSNGATFYNQKFQGRATLTVDTSTSTAYMELSSLRSEDTAVYYCTRSHLLRASWFAYWGQGTLVTVSSASGGGGSGGGGSGGGGSDIVMTQSPDSLAVSLGERATINCKSSQSLLNSGNQKNYLTWYLQKPGQPPKLLIYWASTRESGVPDRFSGSGSGTDFTLTISSVQAEDVAVYYCQNDYSYPYTFGGGTKLEIKAAARGDIVMTQSPDSLAVSLGERATINCKSSQSLLNSRTPKNYLAWYQQKPGQPPKLLIYWASTRKSGVPDRFSGSGSGTDFTLTISSLQAEDVAVYYCKQSYNLLTFGGGTKVEIKGGGGSGGGGSGASAAGGGGSGGGGSQVQLVQSGAEVKKPGASVKVSCKASGYTFTHYYIYWVRQAPGQGLEWMGGVNPSNGGTHFNEKFKSRVTMTRDTSISTAYMELSRLRSDDTAVYYCARSEYDYGLGFAYWGQGTLVTVSSGGGGSHHHHHHHH

SEQ ID NO: 15 - protein, 526 aa, synthetic construct
  source 1..526: note = Targeting module
GQVQLVQSGAEVKKPGASVKMSCKASGYTFTDYYMKWVKQAPGQGLEWIGDIIPSNGATFYNQKFKGRATLTVDKSTSTAYMELSSLRSEDTAVYYCTRSHLLRASWFAYWGQGTLVTVSSASGGGGSGGGGSGGGGSDFVMTQSPDSLAVSLGERATMNCKSSQSLLNSGNQKNYLTWYLQKPGQPPKLLIYWASTRESGVPDRFSGSGSGTDFTLTISSVQAEDVAVYYCQNDYSYPYTFGGGTKLEIKAAARGDIVMTQSPDSLAVSLGERATINCKSSQSLLNSRTPKNYLAWYQQKPGQPPKLLIYWASTRKSGVPDRFSGSGSGTDFTLTISSLQAEDVAVYYCKQSYNLLTFGGGTKVEIKGGGGSGGGGSGASAAGGGGSGGGGSQVQLVQSGAEVKKPGASVKVSCKASGYTFTHYYIYWVRQAPGQGLEWMGGVNPSNGGTHFNEKFKSRVTMTRDTSISTAYMELSRLRSDDTAVYYCARSEYDYGLGFAYWGQGTLVTVSSGGGGSHHHHHHHH

SEQ ID NO: 16 - protein, 525 aa, synthetic construct
  source 1..525: note = Targeting module
EVQLVQSGAEVKKPGASVKMSCKASGYTFTDYYMKWVKQAPGQGLEWIGDIIPSNGATFYNQKFKGRATLTVDRSTSTAYMELSSLRSEDTAVYYCTRSHLLRASWFAYWGQGTLVTVSSASGGGGSGGGGSGGGGSDFVMTQSPDSLAVSLGERATINCESSQSLLNTGNQKNYLTWYLQKPGQPPKLLIYWASTRESGVPDRFSGSGSGTDFTLTISSVQAEDVAVYYCQNDYSYPYTFGGGTKLEIKAAARGDIVMTQSPDSLAVSLGERATINCKSSQSLLNSRTPKNYLAWYQQKPGQPPKLLIYWASTRKSGVPDRFSGSGSGTDFTLTISSLQAEDVAVYYCKQSYNLLTFGGGTKVEIKGGGGSGGGGSGASAAGGGGSGGGGSQVQLVQSGAEVKKPGASVKVSCKASGYTFTHYYIYWVRQAPGQGLEWMGGVNPSNGGTHFNEKFKSRVTMTRDTSISTAYMELSRLRSDDTAVYYCARSEYDYGLGFAYWGQGTLVTVSSGGGGSHHHHHHHH

SEQ ID NO: 17 - protein, 525 aa, synthetic construct
  source 1..525: note = Targeting module
EVQLVQSGAEVKKPGASVKMSCKASGYTFTDYYMKWVKQAPGQGLEWIGDIIPSNGATFYNQKFKGRATLTVDRSTSTAYMELSSLRSEDTAVYYCTRSHLLRASWFAYWGQGTLVTVSSASGGGGSGGGGSGGGGSDFVMTQSPDSLAVSLGERATINCESSQSLLNTGNQKNYLTWYLQKPGQPPKLLIYWASTRESGVPDRFSGSGSGTDFTLTISSVQAEDVAVYYCQNDYSYPYTFGGGTKLEIKAAARGDIVMTQSPDSLAVSLGERVTMNCKSSQSLLNSRTPKNYLAWYQQKPGQSPKLLIYWASTRKSGVPDRFSGSGSGTDFTLTISSVQAEDVAVYYCKQSYNLLTFGGGTKLEIKGGGGSGGGGSGASAAGGGGSGGGGSQVQLVESGAEVVKPGASVKLSCKASGYAFTHYYIYWIKQAPGQGLEWIGGVNPSNGGTHFNEKFKSRATLTVDTSISTAYMELSRLRSDDTAVYYCTRSEYDYGLGFAYWGQGTLVTVSSGGGGSHHHHHHHH

SEQ ID NO: 18 - protein, 33 aa, Saccharomyces cerevisiae
RMKQLEPKVEELLPKNYHLENEVARLKKLVGER

SEQ ID NO: 19 - protein, 14 aa, Saccharomyces cerevisiae
NYHLENEVARLKKL

SEQ ID NO: 20 - protein, 51 aa, Homo sapiens
MDPDLEIRAAFLRQRNTALRTEVAELEQEVQRLENEVSQYETRYGPLGGGK

SEQ ID NO: 21 - protein, 51 aa, Homo sapiens
MDPDLEIEAAFLERENTALETRVAELRQRVQRLRNRVSQYRTRYGPLGGGK

SEQ ID NO: 22 - protein, 10 aa, Homo sapiens
KPLPEVTDEY

SEQ ID NO: 23 - protein, 20 aa, Homo sapiens
  VARIANT 16: note = X can be any amino acid
LEKEALKKIIEDQQEXLNKW

SEQ ID NO: 24 - protein, 20 aa, Homo sapiens
LEKEALKKIIEDQQEALNKW

SEQ ID NO: 25 - protein, 112 aa, synthetic construct
  source 1..112: note = Humanized scFv VL chain
DIVMTQSPDSLAVSLGERATINCRSSQSLLDSRTKKNYLAWYQQKPGQPPKLLIYWASTRESGVPDRFSGSGSGTDFTLTISSLQAEDVAVYYCKQSYNLPTFGGGTKVEIK

SEQ ID NO: 26 - protein, 118 aa, synthetic construct
  source 1..118: note = Humanized scFv VH chain
EVQLVESGGGLVQPGGSLRLSCAASGFTFSDFWMNWVRQAPGKGLEWVGQIRNKPNNYETYYSDSLKGRFTISRDDSKSITYLQMNSLRAEDTAVYYCTLGNSWFAYWGQGTLVTVSS

SEQ ID NO: 27 - protein, 133 aa, synthetic construct
  source 1..133: note = CD28 extracellular hinge domain with mutation
KILVKQSPMLVAYDNAVNLSCKYSYNLFSREFRASLHKGLDSAVEVCVVYGNYSQQLQVYSKTGFNCDGKLGNESVTFYLQNLYVNQTDIYFCKIEVMAPPPALDNEKSNGTIIHVKGKHLCPSPLFPGPSKP

SEQ ID NO: 28 - protein, 27 aa, Homo sapiens
FWVLVVVGGVLACYSLLVTVAFIIFWV

SEQ ID NO: 29 - protein, 21 aa, Homo sapiens
FWLPIGCAAFVVVCILGCILI

SEQ ID NO: 30 - protein, 41 aa, synthetic construct
  source 1..41: note = CD28 intracellular signaling domain with mutations
RSKRSRGGHSDYMNMTPRRPGPTRKHYQPYAPPRDFAAYRS

SEQ ID NO: 31 - protein, 41 aa, synthetic construct
  source 1..41: note = CD28 intracellular signaling domain with mutations
RSKRSRGGHSDYMFMTPRRPGPTRKHYQPYAPPRDFAAYRS

SEQ ID NO: 32 - protein, 109 aa, Homo sapiens
FSRSADAPAYQQGQNQLYNELNLGRREEYDVLDKRRGRDPEMGGKPRRKNPQEGLYNELQKDKMAEAYSEIGMKGERRRGKGHDGLYQGLSTATKDTYDALHMQALPPR

SEQ ID NO: 33 - protein, 109 aa, synthetic construct
  source 1..109: note = CD3zeta intracellular signaling domain with mutation
FSRSADAPAYQQGQNQLYNELNLGRREEYDVLDKRRGRDPEMGGKPRRKNPQEGLYNELQKDKMAEAYSEIGMKGERRRGKGHDGLYQGLSTATKDTYGALHMQALPPR

SEQ ID NO: 34 - protein, 112 aa, synthetic construct
  source 1..112: note = CD3zeta intracellular signaling domain with mutations
RVKFSRSADAPAYQQGQNQLYNELNLGRREEYDVLDKRRGRDPEMGGKPRRKNPQEGLYNELQKDKMAEAYSEIGMKGERRRGKGHDGLYQGLSTATKDTYDAYRHQALPPR

SEQ ID NO: 35 - protein, 38 aa, Homo sapiens
CWLTKKKYSSSVHDPNGEYMFMRAVNTAKKSRLTDVTL

SEQ ID NO: 36 - protein, 42 aa, Homo sapiens
KRGRKKLLYIFKQPFMRPVQTTQEEDGCSCRFPEEEEGGCEL

SEQ ID NO: 37 - protein, 155 aa, synthetic construct
  source 1..155: note = truncated IL-7Ralpha intracellular signaling domain
KKRIKPIVWPSLPDHKKTLEHLCKKPRKNLNVSFNPESFLDCQIHRVDDIQARDEVEGFLQDTFPQQLEESEKQRLGGDVQSPNCPSEDVVIGPHVYQDLLLSLGTTNSTLPPPFSLQSGILTLNPVAQGQPILTSLGSNQEEAYVTMSSFYQNQ

SEQ ID NO: 38 - protein, 94 aa, synthetic construct
  source 1..94: note = truncated IL-2Rbeta intracellular signaling domain
NCRNTGPWLKKVLKCNTPDPSKFFSQLSSEHGGDVQKWLSSPFPSSSFSPGGLAPEISPLEVLERDKVTQLLPLNTDAYLSLQELQGQDPTHLV

SEQ ID NO: 39 - protein, 634 aa, synthetic construct
  source 1..634: note = Humanized switchable chimeric antigen receptor
MRRMQLLLLIALSLALVTNSEFKPLPEVTDEYAAAGPGGGGSKILVKQSPMLVAYDNAVNLSCKYSYNLFSREFRASLHKGLDSAVEVCVVYGNYSQQLQVYSKTGFNCDGKLGNESVTFYLQNLYVNQTDIYFCKIEVMAPPPALDNEKSNGTIIHVKGKHLCPSPLFPGPSKPFWVLVVVGGVLACYSLLVTVAFIIFWVRSKRSRGGHSDYMNMTPRRPGPTRKHYQPYAPPRDFAAYRSGGGGSGGGASGGGGSFSRSADAPAYQQGQNQLYNELNLGRREEYDVLDKRRGRDPEMGGKPRRKNPQEGLYNELQKDKMAEAYSEIGMKGERRRGKGHDGLYQGLSTATKDTYGALHMQALPPRGSGSSGEGRGSLLTCGDVEENPGPPVATMVSKGEELFTGVVPILVELDGDVNGHKFSVSGEGEGDATYGKLTLKFICTTGKLPVPWPTLVTTLTYGVQCFSRYPDHMKQHDFFKSAMPEGYVQERTIFFKDDGNYKTRAEVKFEGDTLVNRIELKGIDFKEDGNILGHKLEYNYNSHNVYIMADKQKNGIKVNFKIRHNIEDGSVQLADHYQQNTPIGDGPVLLPDNHYLSTQSALSKDPNEKRDHMVLLEFVTAAGITLGMDELYK

SEQ ID NO: 40 - protein, 624 aa, synthetic construct
  source 1..624: note = Humanized switchable chimeric antigen receptor
MRRMQLLLLIALSLALVTNSEFKPLPEVTDEYAAAGPGGGGSKILVKQSPMLVAYDNAVNLSCKYSYNLFSREFRASLHKGLDSAVEVCVVYGNYSQQLQVYSKTGFNCDGKLGNESVTFYLQNLYVNQTDIYFCKIEVMAPPPALDNEKSNGTIIHVKGKHLCPSPLFPGPSKPFWVLVVVGGVLACYSLLVTVAFIIFWVRSKRSRGGHSDYMNMTPRRPGPTRKHYQPYAPPRDFAAYRSGGGGSFSRSADAPAYQQGQNQLYNELNLGRREEYDVLDKRRGRDPEMGGKPRRKNPQEGLYNELQKDKMAEAYSEIGMKGERRRGKGHDGLYQGLSTATKDTYDALHMQALPPRGSGSSGEGRGSLLTCGDVEENPGPPVATMVSKGEELFTGVVPILVELDGDVNGHKFSVSGEGEGDATYGKLTLKFICTTGKLPVPWPTLVTTLTYGVQCFSRYPDHMKQHDFFKSAMPEGYVQERTIFFKDDGNYKTRAEVKFEGDTLVNRIELKGIDFKEDGNILGHKLEYNYNSHNVYIMADKQKNGIKVNFKIRHNIEDGSVQLADHYQQNTPIGDGPVLLPDNHYLSTQSALSKDPNEKRDHMVLLEFVTAAGITLGMDELYK

SEQ ID NO: 41 - protein, 671 aa, synthetic construct
  source 1..671: note = Humanized switchable chimeric antigen receptor
MRRMQLLLLIALSLALVTNSEFKPLPEVTDEYAAAGPGGGGSKILVKQSPMLVAYDNAVNLSCKYSYNLFSREFRASLHKGLDSAVEVCVVYGNYSQQLQVYSKTGFNCDGKLGNESVTFYLQNLYVNQTDIYFCKIEVMAPPPALDNEKSNGTIIHVKGKHLCPSPLFPGPSKPFWVLVVVGGVLACYSLLVTVAFIIFWVRSKRSRGGHSDYMNMTPRRPGPTRKHYQPYAPPRDFAAYRSGGGGSKRGRKKLLYIFKQPFMRPVQTTQEEDGCSCRFPEEEEGGCELGGGGSFSRSADAPAYQQGQNQLYNELNLGRREEYDVLDKRRGRDPEMGGKPRRKNPQEGLYNELQKDKMAEAYSEIGMKGERRRGKGHDGLYQGLSTATKDTYDALHMQALPPRGSGSSGEGRGSLLTCGDVEENPGPPVATMVSKGEELFTGVVPILVELDGDVNGHKFSVSGEGEGDATYGKLTLKFICTTGKLPVPWPTLVTTLTYGVQCFSRYPDHMKQHDFFKSAMPEGYVQERTIFFKDDGNYKTRAEVKFEGDTLVNRIELKGIDFKEDGNILGHKLEYNYNSHNVYIMADKQKNGIKVNFKIRHNIEDGSVQLADHYQQNTPIGDGPVLLPDNHYLSTQSALSKDPNEKRDHMVLLEFVTAAGITLGMDELYK

SEQ ID NO: 42 - protein, 716 aa, synthetic construct
  source 1..716: note = Humanized switchable chimeric antigen receptor
MRRMQLLLLIALSLALVTNSEFKPLPEVTDEYAAAGPGGGGSKILVKQSPMLVAYDNAVNLSCKYSYNLFSREFRASLHKGLDSAVEVCVVYGNYSQQLQVYSKTGFNCDGKLGNESVTFYLQNLYVNQTDIYFCKIEVMAPPPALDNEKSNGTIIHVKGKHLCPSPLFPGPSKPFWVLVVVGGVLACYSLLVTVAFIIFWVRSKRSRGGHSDYMNMTPRRPGPTRKHYQPYAPPRDFAAYRSNCRNTGPWLKKVLKCNTPDPSKFFSQLSSEHGGDVQKWLSSPFPSSSFSPGGLAPEISPLEVLERDKVTQLLPLNTDAYLSLQELQGQDPTHLVRVKFSRSADAPAYQQGQNQLYNELNLGRREEYDVLDKRRGRDPEMGGKPRRKNPQEGLYNELQKDKMAEAYSEIGMKGERRRGKGHDGLYQGLSTATKDTYDAYRHQALPPRGSGSSGEGRGSLLTCGDVEENPGPPVATMVSKGEELFTGVVPILVELDGDVNGHKFSVSGEGEGDATYGKLTLKFICTTGKLPVPWPTLVTTLTYGVQCFSRYPDHMKQHDFFKSAMPEGYVQERTIFFKDDGNYKTRAEVKFEGDTLVNRIELKGIDFKEDGNILGHKLEYNYNSHNVYIMADKQKNGIKVNFKIRHNIEDGSVQLADHYQQNTPIGDGPVLLPDNHYLSTQSALSKDPNEKRDHMVLLEFVTAAGITLGMDELYK

SEQ ID NO: 43 - protein, 784 aa, synthetic construct
  source 1..784: note = Humanized switchable chimeric antigen receptor
MRRMQLLLLIALSLALVTNSEFKPLPEVTDEYAAAGPGGGGSKILVKQSPMLVAYDNAVNLSCKYSYNLFSREFRASLHKGLDSAVEVCVVYGNYSQQLQVYSKTGFNCDGKLGNESVTFYLQNLYVNQTDIYFCKIEVMAPPPALDNEKSNGTIIHVKGKHLCPSPLFPGPSKPFWVLVVVGGVLACYSLLVTVAFIIFWVRSKRSRGGHSDYMNMTPRRPGPTRKHYQPYAPPRDFAAYRSGGGGSKKRIKPIVWPSLPDHKKTLEHLCKKPRKNLNVSFNPESFLDCQIHRVDDIQARDEVEGFLQDTFPQQLEESEKQRLGGDVQSPNCPSEDVVIGPHVYQDLLLSLGTTNSTLPPPFSLQSGILTLNPVAQGQPILTSLGSNQEEAYVTMSSFYQNQGGGGSFSRSADAPAYQQGQNQLYNELNLGRREEYDVLDKRRGRDPEMGGKPRRKNPQEGLYNELQKDKMAEAYSEIGMKGERRRGKGHDGLYQGLSTATKDTYDALHMQALPPRGSGSSGEGRGSLLTCGDVEENPGPPVATMVSKGEELFTGVVPILVELDGDVNGHKFSVSGEGEGDATYGKLTLKFICTTGKLPVPWPTLVTTLTYGVQCFSRYPDHMKQHDFFKSAMPEGYVQERTIFFKDDGNYKTRAEVKFEGDTLVNRIELKGIDFKEDGNILGHKLEYNYNSHNVYIMADKQKNGIKVNFKIRHNIEDGSVQLADHYQQNTPIGDGPVLLPDNHYLSTQSALSKDPNEKRDHMVLLEFVTAAGITLGMDELYK

SEQ ID NO: 44 - protein, 784 aa, synthetic construct
  source 1..784: note = Humanized switchable chimeric antigen receptor
MRRMQLLLLIALSLALVTNSEFKPLPEVTDEYAAAGPGGGGSKILVKQSPMLVAYDNAVNLSCKYSYNLFSREFRASLHKGLDSAVEVCVVYGNYSQQLQVYSKTGFNCDGKLGNESVTFYLQNLYVNQTDIYFCKIEVMAPPPALDNEKSNGTIIHVKGKHLCPSPLFPGPSKPFWVLVVVGGVLACYSLLVTVAFIIFWVRSKRSRGGHSDYMNMTPRRPGPTRKHYQPYAPPRDFAAYRSGGGGSFSRSADAPAYQQGQNQLYNELNLGRREEYDVLDKRRGRDPEMGGKPRRKNPQEGLYNELQKDKMAEAYSEIGMKGERRRGKGHDGLYQGLSTATKDTYDALHMQALPPRGGGGSKKRIKPIVWPSLPDHKKTLEHLCKKPRKNLNVSFNPESFLDCQIHRVDDIQARDEVEGFLQDTFPQQLEESEKQRLGGDVQSPNCPSEDVVIGPHVYQDLLLSLGTTNSTLPPPFSLQSGILTLNPVAQGQPILTSLGSNQEEAYVTMSSFYQNQGSGSSGEGRGSLLTCGDVEENPGPPVATMVSKGEELFTGVVPILVELDGDVNGHKFSVSGEGEGDATYGKLTLKFICTTGKLPVPWPTLVTTLTYGVQCFSRYPDHMKQHDFFKSAMPEGYVQERTIFFKDDGNYKTRAEVKFEGDTLVNRIELKGIDFKEDGNILGHKLEYNYNSHNVYIMADKQKNGIKVNFKIRHNIEDGSVQLADHYQQNTPIGDGPVLLPDNHYLSTQSALSKDPNEKRDHMVLLEFVTAAGITLGMDELYK

SEQ ID NO: 45 - protein, 624 aa, synthetic construct
  source 1..624: note = Humanized switchable chimeric antigen receptor
MRRMQLLLLIALSLALVTNSEFKPLPEVTDEYAAAGPGGGGSKILVKQSPMLVAYDNAVNLSCKYSYNLFSREFRASLHKGLDSAVEVCVVYGNYSQQLQVYSKTGFNCDGKLGNESVTFYLQNLYVNQTDIYFCKIEVMAPPPALDNEKSNGTIIHVKGKHLCPSPLFPGPSKPFWVLVVVGGVLACYSLLVTVAFIIFWVRSKRSRGGHSDYMFMTPRRPGPTRKHYQPYAPPRDFAAYRSGGGGSFSRSADAPAYQQGQNQLYNELNLGRREEYDVLDKRRGRDPEMGGKPRRKNPQEGLYNELQKDKMAEAYSEIGMKGERRRGKGHDGLYQGLSTATKDTYDALHMQALPPRGSGSSGEGRGSLLTCGDVEENPGPPVATMVSKGEELFTGVVPILVELDGDVNGHKFSVSGEGEGDATYGKLTLKFICTTGKLPVPWPTLVTTLTYGVQCFSRYPDHMKQHDFFKSAMPEGYVQERTIFFKDDGNYKTRAEVKFEGDTLVNRIELKGIDFKEDGNILGHKLEYNYNSHNVYIMADKQKNGIKVNFKIRHNIEDGSVQLADHYQQNTPIGDGPVLLPDNHYLSTQSALSKDPNEKRDHMVLLEFVTAAGITLGMDELYK

SEQ ID NO: 46 - protein, 662 aa, synthetic construct
  source 1..662: note = Humanized switchable chimeric antigen receptor
MRRMQLLLLIALSLALVTNSEFKPLPEVTDEYAAAGPGGGGSKILVKQSPMLVAYDNAVNLSCKYSYNLFSREFRASLHKGLDSAVEVCVVYGNYSQQLQVYSKTGFNCDGKLGNESVTFYLQNLYVNQTDIYFCKIEVMAPPPALDNEKSNGTIIHVKGKHLCPSPLFPGPSKPFWLPIGCAAFVVVCILGCILICWLTKKKYSSSVHDPNGEYMFMRAVNTAKKSRLTDVTLGGGGSKRGRKKLLYIFKQPFMRPVQTTQEEDGCSCRFPEEEEGGCELGGGGSFSRSADAPAYQQGQNQLYNELNLGRREEYDVLDKRRGRDPEMGGKPRRKNPQEGLYNELQKDKMAEAYSEIGMKGERRRGKGHDGLYQGLSTATKDTYDALHMQALPPRGSGSSGEGRGSLLTCGDVEENPGPPVATMVSKGEELFTGVVPILVELDGDVNGHKFSVSGEGEGDATYGKLTLKFICTTGKLPVPWPTLVTTLTYGVQCFSRYPDHMKQHDFFKSAMPEGYVQERTIFFKDDGNYKTRAEVKFEGDTLVNRIELKGIDFKEDGNILGHKLEYNYNSHNVYIMADKQKNGIKVNFKIRHNIEDGSVQLADHYQQNTPIGDGPVLLPDNHYLSTQSALSKDPNEKRDHMVLLEFVTAAGITLGMDELYK

SEQ ID NO: 47 - protein, 615 aa, synthetic construct
  source 1..615: note = Humanized switchable chimeric antigen receptor
MRRMQLLLLIALSLALVTNSEFKPLPEVTDEYAAAGPGGGGSKILVKQSPMLVAYDNAVNLSCKYSYNLFSREFRASLHKGLDSAVEVCVVYGNYSQQLQVYSKTGFNCDGKLGNESVTFYLQNLYVNQTDIYFCKIEVMAPPPALDNEKSNGTIIHVKGKHLCPSPLFPGPSKPFWLPIGCAAFVVVCILGCILICWLTKKKYSSSVHDPNGEYMFMRAVNTAKKSRLTDVTLGGGGSFSRSADAPAYQQGQNQLYNELNLGRREEYDVLDKRRGRDPEMGGKPRRKNPQEGLYNELQKDKMAEAYSEIGMKGERRRGKGHDGLYQGLSTATKDTYDALHMQALPPRGSGSSGEGRGSLLTCGDVEENPGPPVATMVSKGEELFTGVVPILVELDGDVNGHKFSVSGEGEGDATYGKLTLKFICTTGKLPVPWPTLVTTLTYGVQCFSRYPDHMKQHDFFKSAMPEGYVQERTIFFKDDGNYKTRAEVKFEGDTLVNRIELKGIDFKEDGNILGHKLEYNYNSHNVYIMADKQKNGIKVNFKIRHNIEDGSVQLADHYQQNTPIGDGPVLLPDNHYLSTQSALSKDPNEKRDHMVLLEFVTAAGITLGMDELYK

SEQ ID NO: 48 - protein, 894 aa, synthetic construct
  source 1..894: note = Humanized switchable chimeric antigen receptor
MRRMQLLLLIALSLALVTNSEFQVQLVQSGAEVKKPGASVKVSCKASGYTFTHYYIYWVRQAPGQGLEWMGGVNPSNGGTHFNEKFKSRVTMTRDTSISTAYMELSRLRSDDTAVYYCARSEYDYGLGFAYWGQGTLVTVSSGGGGSGGGGSGGGGSDIVMTQSPDSLAVSLGERATINCKSSQSLLNSRTPKNYLAWYQQKPGQPPKLLIYWASTRKSGVPDRFSGSGSGTDFTLTISSLQAEDVAVYYCKQSYNLLTFGGGTKVEIKAAALEKEALKKIIEDQQEALNKWAAAGPGGGGSKILVKQSPMLVAYDNAVNLSCKYSYNLFSREFRASLHKGLDSAVEVCVVYGNYSQQLQVYSKTGFNCDGKLGNESVTFYLQNLYVNQTDIYFCKIEVMAPPPALDNEKSNGTIIHVKGKHLCPSPLFPGPSKPFWVLVVVGGVLACYSLLVTVAFIIFWVRSKRSRGGHSDYMNMTPRRPGPTRKHYQPYAPPRDFAAYRSGGGGSGGGASGGGGSFSRSADAPAYQQGQNQLYNELNLGRREEYDVLDKRRGRDPEMGGKPRRKNPQEGLYNELQKDKMAEAYSEIGMKGERRRGKGHDGLYQGLSTATKDTYGALHMQALPPRGSGSSGEGRGSLLTCGDVEENPGPPVATMVSKGEELFTGVVPILVELDGDVNGHKFSVSGEGEGDATYGKLTLKFICTTGKLPVPWPTLVTTLTYGVQCFSRYPDHMKQHDFFKSAMPEGYVQERTIFFKDDGNYKTRAEVKFEGDTLVNRIELKGIDFKEDGNILGHKLEYNYNSHNVYIMADKQKNGIKVNFKIRHNIEDGSVQLADHYQQNTPIGDGPVLLPDNHYLSTQSALSKDPNEKRDHMVLLEFVTAAGITLGMDELYK

SEQ ID NO: 49 - protein, 884 aa, synthetic construct
  source 1..884: note = Humanized switchable chimeric antigen receptor
MRRMQLLLLIALSLALVTNSEFQVQLVQSGAEVKKPGASVKVSCKASGYTFTHYYIYWVRQAPGQGLEWMGGVNPSNGGTHFNEKFKSRVTMTRDTSISTAYMELSRLRSDDTAVYYCARSEYDYGLGFAYWGQGTLVTVSSGGGGSGGGGSGGGGSDIVMTQSPDSLAVSLGERATINCKSSQSLLNSRTPKNYLAWYQQKPGQPPKLLIYWASTRKSGVPDRFSGSGSGTDFTLTISSLQAEDVAVYYCKQSYNLLTFGGGTKVEIKAAALEKEALKKIIEDQQEALNKWAAAGPGGGGSKILVKQSPMLVAYDNAVNLSCKYSYNLFSREFRASLHKGLDSAVEVCVVYGNYSQQLQVYSKTGFNCDGKLGNESVTFYLQNLYVNQTDIYFCKIEVMAPPPALDNEKSNGTIIHVKGKHLCPSPLFPGPSKPFWVLVVVGGVLACYSLLVTVAFIIFWVRSKRSRGGHSDYMNMTPRRPGPTRKHYQPYAPPRDFAAYRSGGGGSFSRSADAPAYQQGQNQLYNELNLGRREEYDVLDKRRGRDPEMGGKPRRKNPQEGLYNELQKDKMAEAYSEIGMKGERRRGKGHDGLYQGLSTATKDTYDALHMQALPPRGSGSSGEGRGSLLTCGDVEENPGPPVATMVSKGEELFTGVVPILVELDGDVNGHKFSVSGEGEGDATYGKLTLKFICTTGKLPVPWPTLVTTLTYGVQCFSRYPDHMKQHDFFKSAMPEGYVQERTIFFKDDGNYKTRAEVKFEGDTLVNRIELKGIDFKEDGNILGHKLEYNYNSHNVYIMADKQKNGIKVNFKIRHNIEDGSVQLADHYQQNTPIGDGPVLLPDNHYLSTQSALSKDPNEKRDHMVLLEFVTAAGITLGMDELYK

SEQ ID NO: 50 - protein, 931 aa, synthetic construct
  source 1..931: note = Humanized switchable chimeric antigen receptor
MRRMQLLLLIALSLALVTNSEFQVQLVQSGAEVKKPGASVKVSCKASGYTFTHYYIYWVRQAPGQGLEWMGGVNPSNGGTHFNEKFKSRVTMTRDTSISTAYMELSRLRSDDTAVYYCARSEYDYGLGFAYWGQGTLVTVSSGGGGSGGGGSGGGGSDIVMTQSPDSLAVSLGERATINCKSSQSLLNSRTPKNYLAWYQQKPGQPPKLLIYWASTRKSGVPDRFSGSGSGTDFTLTISSLQAEDVAVYYCKQSYNLLTFGGGTKVEIKAAALEKEALKKIIEDQQEALNKWAAAGPGGGGSKILVKQSPMLVAYDNAVNLSCKYSYNLFSREFRASLHKGLDSAVEVCVVYGNYSQQLQVYSKTGFNCDGKLGNESVTFYLQNLYVNQTDIYFCKIEVMAPPPALDNEKSNGTIIHVKGKHLCPSPLFPGPSKPFWVLVVVGGVLACYSLLVTVAFIIFWVRSKRSRGGHSDYMNMTPRRPGPTRKHYQPYAPPRDFAAYRSGGGGSKRGRKKLLYIFKQPFMRPVQTTQEEDGCSCRFPEEEEGGCELGGGGSFSRSADAPAYQQGQNQLYNELNLGRREEYDVLDKRRGRDPEMGGKPRRKNPQEGLYNELQKDKMAEAYSEIGMKGERRRGKGHDGLYQGLSTATKDTYDALHMQALPPRGSGSSGEGRGSLLTCGDVEENPGPPVATMVSKGEELFTGVVPILVELDGDVNGHKFSVSGEGEGDATYGKLTLKFICTTGKLPVPWPTLVTTLTYGVQCFSRYPDHMKQHDFFKSAMPEGYVQERTIFFKDDGNYKTRAEVKFEGDTLVNRIELKGIDFKEDGNILGHKLEYNYNSHNVYIMADKQKNGIKVNFKIRHNIEDGSVQLADHYQQNTPIGDGPVLLPDNHYLSTQSALSKDPNEKRDHMVLLEFVTAAGITLGMDELYK

SEQ ID NO: 51 - protein, 976 aa, synthetic construct
  source 1..976: note = Humanized switchable chimeric antigen receptor
MRRMQLLLLIALSLALVTNSEFQVQLVQSGAEVKKPGASVKVSCKASGYTFTHYYIYWVRQAPGQGLEWMGGVNPSNGGTHFNEKFKSRVTMTRDTSISTAYMELSRLRSDDTAVYYCARSEYDYGLGFAYWGQGTLVTVSSGGGGSGGGGSGGGGSDIVMTQSPDSLAVSLGERATINCKSSQSLLNSRTPKNYLAWYQQKPGQPPKLLIYWASTRKSGVPDRFSGSGSGTDFTLTISSLQAEDVAVYYCKQSYNLLTFGGGTKVEIKAAALEKEALKKIIEDQQEALNKWAAAGPGGGGSKILVKQSPMLVAYDNAVNLSCKYSYNLFSREFRASLHKGLDSAVEVCVVYGNYSQQLQVYSKTGFNCDGKLGNESVTFYLQNLYVNQTDIYFCKIEVMAPPPALDNEKSNGTIIHVKGKHLCPSPLFPGPSKPFWVLVVVGGVLACYSLLVTVAFIIFWVRSKRSRGGHSDYMNMTPRRPGPTRKHYQPYAPPRDFAAYRSNCRNTGPWLKKVLKCNTPDPSKFFSQLSSEHGGDVQKWLSSPFPSSSFSPGGLAPEISPLEVLERDKVTQLLPLNTDAYLSLQELQGQDPTHLVRVKFSRSADAPAYQQGQNQLYNELNLGRREEYDVLDKRRGRDPEMGGKPRRKNPQEGLYNELQKDKMAEAYSEIGMKGERRRGKGHDGLYQGLSTATKDTYDAYRHQALPPRGSGSSGEGRGSLLTCGDVEENPGPPVATMVSKGEELFTGVVPILVELDGDVNGHKFSVSGEGEGDATYGKLTLKFICTTGKLPVPWPTLVTTLTYGVQCFSRYPDHMKQHDFFKSAMPEGYVQERTIFFKDDGNYKTRAEVKFEGDTLVNRIELKGIDFKEDGNILGHKLEYNYNSHNVYIMADKQKNGIKVNFKIRHNIEDGSVQLADHYQQNTPIGDGPVLLPDNHYLSTQSALSKDPNEKRDHMVLLEFVTAAGITLGMDELYK

SEQ ID NO: 52 - protein, 1044 aa, synthetic construct
  source 1..1044: note = Humanized switchable chimeric antigen receptor
MRRMQLLLLIALSLALVTNSEFQVQLVQSGAEVKKPGASVKVSCKASGYTFTHYYIYWVRQAPGQGLEWMGGVNPSNGGTHFNEKFKSRVTMTRDTSISTAYMELSRLRSDDTAVYYCARSEYDYGLGFAYWGQGTLVTVSSGGGGSGGGGSGGGGSDIVMTQSPDSLAVSLGERATINCKSSQSLLNSRTPKNYLAWYQQKPGQPPKLLIYWASTRKSGVPDRFSGSGSGTDFTLTISSLQAEDVAVYYCKQSYNLLTFGGGTKVEIKAAALEKEALKKIIEDQQEALNKWAAAGPGGGGSKILVKQSPMLVAYDNAVNLSCKYSYNLFSREFRASLHKGLDSAVEVCVVYGNYSQQLQVYSKTGFNCDGKLGNESVTFYLQNLYVNQTDIYFCKIEVMAPPPALDNEKSNGTIIHVKGKHLCPSPLFPGPSKPFWVLVVVGGVLACYSLLVTVAFIIFWVRSKRSRGGHSDYMNMTPRRPGPTRKHYQPYAPPRDFAAYRSGGGGSKKRIKPIVWPSLPDHKKTLEHLCKKPRKNLNVSFNPESFLDCQIHRVDDIQARDEVEGFLQDTFPQQLEESEKQRLGGDVQSPNCPSEDVVIGPHVYQDLLLSLGTTNSTLPPPFSLQSGILTLNPVAQGQPILTSLGSNQEEAYVTMSSFYQNQGGGGSFSRSADAPAYQQGQNQLYNELNLGRREEYDVLDKRRGRDPEMGGKPRRKNPQEGLYNELQKDKMAEAYSEIGMKGERRRGKGHDGLYQGLSTATKDTYDALHMQALPPRGSGSSGEGRGSLLTCGDVEENPGPPVATMVSKGEELFTGVVPILVELDGDVNGHKFSVSGEGEGDATYGKLTLKFICTTGKLPVPWPTLVTTLTYGVQCFSRYPDHMKQHDFFKSAMPEGYVQERTIFFKDDGNYKTRAEVKFEGDTLVNRIELKGIDFKEDGNILGHKLEYNYNSHNVYIMADKQKNGIKVNFKIRHNIEDGSVQLADHYQQNTPIGDGPVLLPDNHYLSTQSALSKDPNEKRDHMVLLEFVTAAGITLGMDELYK

SEQ ID NO: 53 - protein, 1044 aa, synthetic construct
  source 1..1044: note = Humanized switchable chimeric antigen receptor
MRRMQLLLLIALSLALVTNSEFQVQLVQSGAEVKKPGASVKVSCKASGYTFTHYYIYWVRQAPGQGLEWMGGVNPSNGGTHFNEKFKSRVTMTRDTSISTAYMELSRLRSDDTAVYYCARSEYDYGLGFAYWGQGTLVTVSSGGGGSGGGGSGGGGSDIVMTQSPDSLAVSLGERATINCKSSQSLLNSRTPKNYLAWYQQKPGQPPKLLIYWASTRKSGVPDRFSGSGSGTDFTLTISSLQAEDVAVYYCKQSYNLLTFGGGTKVEIKAAALEKEALKKIIEDQQEALNKWAAAGPGGGGSKILVKQSPMLVAYDNAVNLSCKYSYNLFSREFRASLHKGLDSAVEVCVVYGNYSQQLQVYSKTGFNCDGKLGNESVTFYLQNLYVNQTDIYFCKIEVMAPPPALDNEKSNGTIIHVKGKHLCPSPLFPGPSKPFWVLVVVGGVLACYSLLVTVAFIIFWVRSKRSRGGHSDYMNMTPRRPGPTRKHYQPYAPPRDFAAYRSGGGGSFSRSADAPAYQQGQNQLYNELNLGRREEYDVLDKRRGRDPEMGGKPRRKNPQEGLYNELQKDKMAEAYSEIGMKGERRRGKGHDGLYQGLSTATKDTYDALHMQALPPRGGGGSKKRIKPIVWPSLPDHKKTLEHLCKKPRKNLNVSFNPESFLDCQIHRVDDIQARDEVEGFLQDTFPQQLEESEKQRLGGDVQSPNCPSEDVVIGPHVYQDLLLSLGTTNSTLPPPFSLQSGILTLNPVAQGQPILTSLGSNQEEAYVTMSSFYQNQGSGSSGEGRGSLLTCGDVEENPGPPVATMVSKGEELFTGVVPILVELDGDVNGHKFSVSGEGEGDATYGKLTLKFICTTGKLPVPWPTLVTTLTYGVQCFSRYPDHMKQHDFFKSAMPEGYVQERTIFFKDDGNYKTRAEVKFEGDTLVNRIELKGIDFKEDGNILGHKLEYNYNSHNVYIMADKQKNGIKVNFKIRHNIEDGSVQLADHYQQNTPIGDGPVLLPDNHYLSTQSALSKDPNEKRDHMVLLEFVTAAGITLGMDELYK

SEQ ID NO: 54 - protein, 884 aa, synthetic construct
  source 1..884: note = Humanized switchable chimeric antigen receptor
MRRMQLLLLIALSLALVTNSEFQVQLVQSGAEVKKPGASVKVSCKASGYTFTHYYIYWVRQAPGQGLEWMGGVNPSNGGTHFNEKFKSRVTMTRDTSISTAYMELSRLRSDDTAVYYCARSEYDYGLGFAYWGQGTLVTVSSGGGGSGGGGSGGGGSDIVMTQSPDSLAVSLGERATINCKSSQSLLNSRTPKNYLAWYQQKPGQPPKLLIYWASTRKSGVPDRFSGSGSGTDFTLTISSLQAEDVAVYYCKQSYNLLTFGGGTKVEIKAAALEKEALKKIIEDQQEALNKWAAAGPGGGGSKILVKQSPMLVAYDNAVNLSCKYSYNLFSREFRASLHKGLDSAVEVCVVYGNYSQQLQVYSKTGFNCDGKLGNESVTFYLQNLYVNQTDIYFCKIEVMAPPPALDNEKSNGTIIHVKGKHLCPSPLFPGPSKPFWVLVVVGGVLACYSLLVTVAFIIFWVRSKRSRGGHSDYMFMTPRRPGPTRKHYQPYAPPRDFAAYRSGGGGSFSRSADAPAYQQGQNQLYNELNLGRREEYDVLDKRRGRDPEMGGKPRRKNPQEGLYNELQKDKMAEAYSEIGMKGERRRGKGHDGLYQGLSTATKDTYDALHMQALPPRGSGSSGEGRGSLLTCGDVEENPGPPVATMVSKGEELFTGVVPILVELDGDVNGHKFSVSGEGEGDATYGKLTLKFICTTGKLPVPWPTLVTTLTYGVQCFSRYPDHMKQHDFFKSAMPEGYVQERTIFFKDDGNYKTRAEVKFEGDTLVNRIELKGIDFKEDGNILGHKLEYNYNSHNVYIMADKQKNGIKVNFKIRHNIEDGSVQLADHYQQNTPIGDGPVLLPDNHYLSTQSALSKDPNEKRDHMVLLEFVTAAGITLGMDELYK

SEQ ID NO: 55 - protein, 922 aa, synthetic construct
  source 1..922: note = Humanized switchable chimeric antigen receptor
MRRMQLLLLIALSLALVTNSEFQVQLVQSGAEVKKPGASVKVSCKASGYTFTHYYIYWVRQAPGQGLEWMGGVNPSNGGTHFNEKFKSRVTMTRDTSISTAYMELSRLRSDDTAVYYCARSEYDYGLGFAYWGQGTLVTVSSGGGGSGGGGSGGGGSDIVMTQSPDSLAVSLGERATINCKSSQSLLNSRTPKNYLAWYQQKPGQPPKLLIYWASTRKSGVPDRFSGSGSGTDFTLTISSLQAEDVAVYYCKQSYNLLTFGGGTKVEIKAAALEKEALKKIIEDQQEALNKWAAAGPGGGGSKILVKQSPMLVAYDNAVNLSCKYSYNLFSREFRASLHKGLDSAVEVCVVYGNYSQQLQVYSKTGFNCDGKLGNESVTFYLQNLYVNQTDIYFCKIEVMAPPPALDNEKSNGTIIHVKGKHLCPSPLFPGPSKPFWLPIGCAAFVVVCILGCILICWLTKKKYSSSVHDPNGEYMFMRAVNTAKKSRLTDVTLGGGGSKRGRKKLLYIFKQPFMRPVQTTQEEDGCSCRFPEEEEGGCELGGGGSFSRSADAPAYQQGQNQLYNELNLGRREEYDVLDKRRGRDPEMGGKPRRKNPQEGLYNELQKDKMAEAYSEIGMKGERRRGKGHDGLYQGLSTATKDTYDALHMQALPPRGSGSSGEGRGSLLTCGDVEENPGPPVATMVSKGEELFTGVVPILVELDGDVNGHKFSVSGEGEGDATYGKLTLKFICTTGKLPVPWPTLVTTLTYGVQCFSRYPDHMKQHDFFKSAMPEGYVQERTIFFKDDGNYKTRAEVKFEGDTLVNRIELKGIDFKEDGNILGHKLEYNYNSHNVYIMADKQKNGIKVNFKIRHNIEDGSVQLADHYQQNTPIGDGPVLLPDNHYLSTQSALSKDPNEKRDHMVLLEFVTAAGITLGMDELYK

SEQ ID NO: 56 - protein, 875 aa, synthetic construct
  source 1..875: note = Humanized switchable chimeric antigen receptor
MRRMQLLLLIALSLALVTNSEFQVQLVQSGAEVKKPGASVKVSCKASGYTFTHYYIYWVRQAPGQGLEWMGGVNPSNGGTHFNEKFKSRVTMTRDTSISTAYMELSRLRSDDTAVYYCARSEYDYGLGFAYWGQGTLVTVSSGGGGSGGGGSGGGGSDIVMTQSPDSLAVSLGERATINCKSSQSLLNSRTPKNYLAWYQQKPGQPPKLLIYWASTRKSGVPDRFSGSGSGTDFTLTISSLQAEDVAVYYCKQSYNLLTFGGGTKVEIKAAALEKEALKKIIEDQQEALNKWAAAGPGGGGSKILVKQSPMLVAYDNAVNLSCKYSYNLFSREFRASLHKGLDSAVEVCVVYGNYSQQLQVYSKTGFNCDGKLGNESVTFYLQNLYVNQTDIYFCKIEVMAPPPALDNEKSNGTIIHVKGKHLCPSPLFPGPSKPFWLPIGCAAFVVVCILGCILICWLTKKKYSSSVHDPNGEYMFMRAVNTAKKSRLTDVTLGGGGSFSRSADAPAYQQGQNQLYNELNLGRREEYDVLDKRRGRDPEMGGKPRRKNPQEGLYNELQKDKMAEAYSEIGMKGERRRGKGHDGLYQGLSTATKDTYDALHMQALPPRGSGSSGEGRGSLLTCGDVEENPGPPVATMVSKGEELFTGVVPILVELDGDVNGHKFSVSGEGEGDATYGKLTLKFICTTGKLPVPWPTLVTTLTYGVQCFSRYPDHMKQHDFFKSAMPEGYVQERTIFFKDDGNYKTRAEVKFEGDTLVNRIELKGIDFKEDGNILGHKLEYNYNSHNVYIMADKQKNGIKVNFKIRHNIEDGSVQLADHYQQNTPIGDGPVLLPDNHYLSTQSALSKDPNEKRDHMVLLEFVTAAGITLGMDELYK